European Patent Application EP 4 438 619 A1, published October 2, 2024. Title: FUSION PROTEIN, AND PREPARATION METHOD THEREFOR AND USE THEREOF. Applicant: SUN YAT-SEN UNIVERSITY CANCER CENTER (SYSUCC). The sequence listing filed with the application follows.

SEQUENCE LISTING (10 sequences)

SEQ ID NO: 1 - protein, 496 aa, Artificial Sequence
MFAKATRNFLREVDADGDLIAVSNLNDSDKLQLLSLVTKKKRFWCWQRPKYQFLSLTLGDVLIEDQFPSPVVVESDFVKYEGKFANHVSGTLETALGKVKLNLGGSSRVESQSSFGTLRKQEVDLQQLIRDSAERTINLRNPVLQQVLEGRNEVLCVLTQKITTMQKCVISEHMQVEEKCGGIVGIQTKTVQVSATEDGNVTKDSNVVLEIPAATTIAYGVIELYVKLDGQFEFCLLRGKQGGFENKKRIDSVYLDPLVFREFAFIDMPDAAHGISSQDGPLSVLKQATLLLERNFHPFAELPEPQQTALSDIFQAVLFDDELLMVLEPVCDDLVSGLSPTVAVLGELKPRQQQDLVAFLQLVGCSLQGGCPGPEDAGSKQLFMTAYFLVSALAEMPDSAAALLGTCCKLQIIPTLCHLLRALSDDGVSDLEDPTLTPLKDTERFGIVQRLFASADISLERLKSSVKAVILKDSKVFPLLLCITLNGLCALGREHS

SEQ ID NO: 2 - protein, 495 aa, Artificial Sequence
MFAKATRNFLREVDADGDLIAVSNLNDSDKLQLLSLVTKKKRFWCWQRPKYQFLSLTLGDVLIEDQFPSPVVVESDFVKYEGKFANHVSGTLETALGKVKLNLGGSSRVESQSSFGTLRKQEVDLQQLIRDSAERTINLRNPVLQQVLEGRNEVLCVLTQKITTMQKCVISEHMQVEEKCGGIVGIQTKTVQVSATEDGNVTKDSNVVLEIPAATTIAYGVIELYVKLDGQFEFCLLRGKQGGFENKKRIDSVYLDPLVFREFAFIAANLVRGISSQDGPLSVLKQATLLLERNFHPFAELPEPQQTALSDIFQAVLFDDELLMVLEPVCDDLVSGLSPTVAVLGELKPRQQQDLVAFLQLVGCSLQGGCPGPEDAGSKQLFMTAYFLVSALAEMPDSAAALLGTCCKLQIIPTLCHLLRALSDDGVSDLEDPTLTPLKDTERFGIVQRLFASADISLERLKSSVKAVILKDSKVFPLLLCITLNGLCALGREHS

SEQ ID NO: 3 - protein, 511 aa, Artificial Sequence
HHHHHHHHHHHHHHHHMFAKATRNFLREVDADGDLIAVSNLNDSDKLQLLSLVTKKKRFWCWQRPKYQFLSLTLGDVLIEDQFPSPVVVESDFVKYEGKFANHVSGTLETALGKVKLNLGGSSRVESQSSFGTLRKQEVDLQQLIRDSAERTINLRNPVLQQVLEGRNEVLCVLTQKITTMQKCVISEHMQVEEKCGGIVGIQTKTVQVSATEDGNVTKDSNVVLEIPAATTIAYGVIELYVKLDGQFEFCLLRGKQGGFENKKRIDSVYLDPLVFREFAFIAANLVRGISSQDGPLSVLKQATLLLERNFHPFAELPEPQQTALSDIFQAVLFDDELLMVLEPVCDDLVSGLSPTVAVLGELKPRQQQDLVAFLQLVGCSLQGGCPGPEDAGSKQLFMTAYFLVSALAEMPDSAAALLGTCCKLQIIPTLCHLLRALSDDGVSDLEDPTLTPLKDTERFGIVQRLFASADISLERLKSSVKAVILKDSKVFPLLLCITLNGLCALGREHS

SEQ ID NO: 4 - protein, 741 aa, Artificial Sequence
DIQMTQSPSSLSASVGDRVTITCRASQDVNTAVAWYQQKPGKAPKLLIYSASFLYSGVPSRFSGSRSGTDFTLTISSLQPEDFATYYCQQHYTTPPTFGQGTKVEIKRTGSTSGSGKPGSGEGSEVQLVESGGGLVQPGGSLRLSCAASGFNIKDTYIHWVRQAPGKGLEWVARIYPTNGYTRYADSVKGRFTISADTSKNTAYLQMNSLRAEDTAVYYCSRWGGDGFYAMDVWGQGTLVTVSSGSMFAKATRNFLREVDADGDLIAVSNLNDSDKLQLLSLVTKKKRFWCWQRPKYQFLSLTLGDVLIEDQFPSPVVVESDFVKYEGKFANHVSGTLETALGKVKLNLGGSSRVESQSSFGTLRKQEVDLQQLIRDSAERTINLRNPVLQQVLEGRNEVLCVLTQKITTMQKCVISEHMQVEEKCGGIVGIQTKTVQVSATEDGNVTKDSNVVLEIPAATTIAYGVIELYVKLDGQFEFCLLRGKQGGFENKKRIDSVYLDPLVFREFAFIAANLVRGISSQDGPLSVLKQATLLLERNFHPFAELPEPQQTALSDIFQAVLFDDELLMVLEPVCDDLVSGLSPTVAVLGELKPRQQQDLVAFLQLVGCSLQGGCPGPEDAGSKQLFMTAYFLVSALAEMPDSAAALLGTCCKLQIIPTLCHLLRALSDDGVSDLEDPTLTPLKDTERFGIVQRLFASADISLERLKSSVKAVILKDSKVFPLLLCITLNGLCALGREHS

SEQ ID NO: 5 - protein, 266 aa, Artificial Sequence
MFAKATRNFLREVDADGDLIAVSNLNDSDKLQLLSLVTKKKRFWAWQRPKYQFLSLTLGDVLIEDQFPSPVVVESDFVKYEGKFANHVSGTLETALGKVKLNLGGSSRVESQSSFGTLRKQEVDLQQLIRDSAERTINLRNPVLQQVLEGRNEVLAVLTQKITTMQKAVISEHMQVEEKAGGIVGIQTKTVQVSATEDGNVTKDSNVVLEIPAATTIAYGVIELYVKLDGQFEFALLRGKQGGFENKKRIDSVYLDPLVFREFAFI

SEQ ID NO: 6 - protein, 495 aa, Artificial Sequence
MFAKATRNFLREVDADGDLIAVSNLNDSDKLQLLSLVTKKKRFWAWQRPKYQFLSLTLGDVLIEDQFPSPVVVESDFVKYEGKFANHVSGTLETALGKVKLNLGGSSRVESQSSFGTLRKQEVDLQQLIRDSAERTINLRNPVLQQVLEGRNEVLAVLTQKITTMQKAVISEHMQVEEKAGGIVGIQTKTVQVSATEDGNVTKDSNVVLEIPAATTIAYGVIELYVKLDGQFEFALLRGKQGGFENKKRIDSVYLDPLVFREFAFIAANLVRGISSQDGPLSVLKQATLLLERNFHPFAELPEPQQTALSDIFQAVLFDDELLMVLEPVADDLVSGLSPTVAVLGELKPRQQQDLVAFLQLVGASLQGGAPGPEDAGSKQLFMTAYFLVSALAEMPDSAAALLGTAAKLQIIPTLAHLLRALSDDGVSDLEDPTLTPLKDTERFGIVQRLFASADISLERLKSSVKAVILKDSKVFPLLLAITLNGLAALGREHS

SEQ ID NO: 7 - protein, 512 aa, Artificial Sequence
HHHHHHHHHHHHHHHHMFAKATRNFLREVDADGDLIAVSNLNDSDKLQLLSLVTKKKRFWAWQRPKYQFLSLTLGDVLIEDQFPSPVVVESDFVKYEGKFANHVSGTLETALGKVKLNLGGSSRVESQSSFGTLRKQEVDLQQLIRDSAERTINLRNPVLQQVLEGRNEVLAVLTQKITTMQKAVISEHMQVEEKAGGIVGIQTKTVQVSATEDGNVTKDSNVVLEIPAATTIAYGVIELYVKLDGQFEFALLRGKQGGFENKKRIDSVYLDPLVFREFAFIDMPDAAHGISSQDGPLSVLKQATLLLERNFHPFAELPEPQQTALSDIFQAVLFDDELLMVLEPVADDLVSGLSPTVAVLGELKPRQQQDLVAFLQLVGASLQGGAPGPEDAGSKQLFMTAYFLVSALAEMPDSAAALLGTAAKLQIIPTLAHLLRALSDDGVSDLEDPTLTPLKDTERFGIVQRLFASADISLERLKSSVKAVILKDSKVFPLLLAITLNGLAALGREHS

SEQ ID NO: 8 - protein, 511 aa, Artificial Sequence
HHHHHHHHHHHHHHHHMFAKATRNFLREVDADGDLIAVSNLNDSDKLQLLSLVTKKKRFWAWQRPKYQFLSLTLGDVLIEDQFPSPVVVESDFVKYEGKFANHVSGTLETALGKVKLNLGGSSRVESQSSFGTLRKQEVDLQQLIRDSAERTINLRNPVLQQVLEGRNEVLAVLTQKITTMQKAVISEHMQVEEKAGGIVGIQTKTVQVSATEDGNVTKDSNVVLEIPAATTIAYGVIELYVKLDGQFEFALLRGKQGGFENKKRIDSVYLDPLVFREFAFIAANLVRGISSQDGPLSVLKQATLLLERNFHPFAELPEPQQTALSDIFQAVLFDDELLMVLEPVADDLVSGLSPTVAVLGELKPRQQQDLVAFLQLVGASLQGGAPGPEDAGSKQLFMTAYFLVSALAEMPDSAAALLGTAAKLQIIPTLAHLLRALSDDGVSDLEDPTLTPLKDTERFGIVQRLFASADISLERLKSSVKAVILKDSKVFPLLLAITLNGLAALGREHS

SEQ ID NO: 9 - protein, 610 aa, Artificial Sequence
MSDSEVNQEAKPEVKPEVKPETHINLKVSDGSSEIFFKIKKTTPLRRLMEAFAKRQGKEMDSLRFLYDGIRIQADQTPEDLDMEDNDIIEAHREQIGGHHHHHHHHHHHHHHHHMFAKATRNFLREVDADGDLIAVSNLNDSDKLQLLSLVTKKKRFWAWQRPKYQFLSLTLGDVLIEDQFPSPVVVESDFVKYEGKFANHVSGTLETALGKVKLNLGGSSRVESQSSFGTLRKQEVDLQQLIRDSAERTINLRNPVLQQVLEGRNEVLAVLTQKITTMQKAVISEHMQVEEKAGGIVGIQTKTVQVSATEDGNVTKDSNVVLEIPAATTIAYGVIELYVKLDGQFEFALLRGKQGGFENKKRIDSVYLDPLVFREFAFIDMPDAAHGISSQDGPLSVLKQATLLLERNFHPFAELPEPQQTALSDIFQAVLFDDELLMVLEPVADDLVSGLSPTVAVLGELKPRQQQDLVAFLQLVGASLQGGAPGPEDAGSKQLFMTAYFLVSALAEMPDSAAALLGTAAKLQIIPTLAHLLRALSDDGVSDLEDPTLTPLKDTERFGIVQRLFASADISLERLKSSVKAVILKDSKVFPLLLAITLNGLAALGREHS

SEQ ID NO: 10 - protein, 609 aa, Artificial Sequence
MSDSEVNQEAKPEVKPEVKPETHINLKVSDGSSEIFFKIKKTTPLRRLMEAFAKRQGKEMDSLRFLYDGIRIQADQTPEDLDMEDNDIIEAHREQIGGHHHHHHHHHHHHHHHHMFAKATRNFLREVDADGDLIAVSNLNDSDKLQLLSLVTKKKRFWAWQRPKYQFLSLTLGDVLIEDQFPSPVVVESDFVKYEGKFANHVSGTLETALGKVKLNLGGSSRVESQSSFGTLRKQEVDLQQLIRDSAERTINLRNPVLQQVLEGRNEVLAVLTQKITTMQKAVISEHMQVEEKAGGIVGIQTKTVQVSATEDGNVTKDSNVVLEIPAATTIAYGVIELYVKLDGQFEFALLRGKQGGFENKKRIDSVYLDPLVFREFAFIAANLVRGISSQDGPLSVLKQATLLLERNFHPFAELPEPQQTALSDIFQAVLFDDELLMVLEPVADDLVSGLSPTVAVLGELKPRQQQDLVAFLQLVGASLQGGAPGPEDAGSKQLFMTAYFLVSALAEMPDSAAALLGTAAKLQIIPTLAHLLRALSDDGVSDLEDPTLTPLKDTERFGIVQRLFASADISLERLKSSVKAVILKDSKVFPLLLAITLNGLAALGREHS